European Patent Specification EP 3 504 233 B1, published January 17, 2024. Title: Multispecific antibodies facilitating selective light chain pairing. Applicant: Sanofi. The sequence listing filed with the application follows.

SEQUENCE LISTING (33 sequences)

SEQ ID NO: 1 - protein, 112 aa, Artificial Sequence
  mutated MCH2
VIAELPPKVSVFVPPRDGFFGNPRKSKLICQATGFSPRQIQVSWLREGKQVGSGVTTDQVQAEAKESGPTTYKVTSTLTIKESDWLGQSMFTCRVDHRGLTFQQQASSMCVP

SEQ ID NO: 2 - protein, 107 aa, Artificial Sequence
  mutated ECH2
VASRDFTPPTVKILQSSCDGGGHFPPTIQLLCLVSGYTPGTINITWLEDGQVMDVDLSTASTTQEGELASTQSELTLSQKHWLSDRTYTCQVTYQGHTFEDSTKKCA

SEQ ID NO: 3 - protein, 220 aa, Artificial Sequence
  tetravalent spider antibody, light chains A
DIVMTQSPDSLAVSLGERATINCESSQSLLNSGNQKNYLTWYQQKPGQPPKPLIYWASTRESGVPDRFSGSGSGTDFTLTISSLQAEDVAVYYCQNDYSYPYTFGQGTKLEIKRTVAAPSVFIFPPSDEQLKSGTASVVCLLNNFYPREAKVQWKVDNALQSGNSQESVTEQDSKDSTYSLSSTLTLSKADYEKHKVYACEVTHQGLSSPVTKSFNRGEC

SEQ ID NO: 4 - protein, 687 aa, Artificial Sequence
  tetravalent spider antibody, heavy chains
QVQLVQSGAEVKKPGASVKVSCKASGYTFTSYYIHWVRQAPGQGLEWIGCIYPGNVNTNYNEKFKDRATLTVDTSISTAYMELSRLRSDDTAVYFCTRSHYGLDWNFDVWGQGTTVTVSSGGVIAELPPKVSVFVPPRDGFFGNPRKSKLICQATGFSPRQIQVSWLREGKQVGSGVTTDQVQAEAKESGPTTYKVTSTLTIKESDWLGQSMFTCRVDHRGLTFQQNASSMCVPGGGSEVQLVQSGAEVKKPGESLKISCKGSGYSFTDYYMKWARQMPGKGLEWMGDIIPSSGATFYNQKFKGQVTISADKSISTTYLQWSSLKASDTAMYYCARSHLLRASWFAYWGQGTMVTVSSASTKGPSVFPLAPSSKSTSGGTAALGCLVKDYFPEPVTVSWNSGALTSGVHTFPAVLQSSGLYSLSSVVTVPSSSLGTQTYICNVNHKPSNTKVDKKVEPKSCDKTHTCPPCPAPELLGGPSVFLFPPKPKDTLMISRTPEVTCVVVDVSHEDPEVKFNWYVDGVEVHNAKTKPREEQYNSTYRVVSVLTVLHQDWLNGKEYKCKVSNKALPAPIEKTISKAKGQPREPQVYTLPPSRDELTKNQVSLTCLVKGFYPSDIAVEWESNGQPENNYKTTPPVLDSDGSFFLYSKLTVDKSRWQQGNVFSCSVMHEALHNHYTQKSLSLSPG

SEQ ID NO: 5 - protein, 221 aa, Artificial Sequence
  tetravalent spider antibody, light chains B
DIQMTQSPSSLSASVGDRVTITCHASQNIYVWLNWYQQKPGKAPKLLIYKASNLHTGVPSRFSGSGSGTDFTLTISSLQPEDFATYYCQQGQTYPYTFGGGTKVEIKRTVIAELPPKVSVFVPPRDGFFGNPRKSKLICQATGFSPRQIQVSWLREGKQVGSGVTTDQVQAEAKESGPTTYKVTSTLTIKESDWLGQSMFTCRVDHRGLTFQQNASSMCVP

SEQ ID NO: 6 - protein, 226 aa, Artificial Sequence
  bispecific IgG1 antibody, light chain A
DVLMTQTPLSLPVSLGDQASISCRSSQSIVHSNGNTYLEWYLQKPGQSPKLLIYKVSNRFSGVPDRFSGSGSGTDFTLKISRVEAEDLGVYYCFQGSHVPLTFGAGTKLELKRTVIAELPPKVSVFVPPRDGFFGNPRKSKLICQATGFSPRQIQVSWLREGKQVGSGVTTDQVQAEAKESGPTTYKVTSTLTIKESDWLGQSMFTCRVDHRGLTFQQQASSMCVP

SEQ ID NO: 7 - protein, 462 aa, Artificial Sequence
  bispecific IgG1 antibody, heavy chain A
QVQLQQSGPELVKPGASVKMSCKASGFTFTDSVISWVKQRTGQGLEWIGEIYPGSGSIYYNEKFKGKATLTADKSSNTAYMQLRSLTSEDSAVYFCAMRRSYWGQGTLVTVSAASTKGPVIAELPPKVSVFVPPRDGFFGNPRKSKLICQATGFSPRQIQVSWLREGKQVGSGVTTDQVQAEAKESGPTTYKVTSTLTIKESDWLGQSMFTCRVDHRGLTFQQQASSMCVPEPKSADKTHTCPPCPAPELLGGPSVFLFPPKPKDTLMISRTPEVTCVVVDVSHEDPEVKFNWYVDGVEVHNAKTKPREEQYNSTYRVVSVLTVLHQDWLNGKEYKCKVSNKALPAPIEKTISKAKGQPREPQVCTLPPSRDELTKNQVSLSCAVKGFYPSDIAVEWESNGQPENNYKTTPPVLDSDGSFFLVSKLTVDKSRWQQGNVFSCSVMHEALHNHYTQKSLSLSPG

SEQ ID NO: 8 - protein, 214 aa, Artificial Sequence
  bispecific IgG1 antibody, light chain B
DIVLTQSPATLSVTPGDSVSLSCRASQSISNYLHWYQQKSHESPRLLIKYASQSISGIPSRFSGSGSGTDFTLSINSVETEDFGMYFCQQSKSWPRTFGGGTELEIKRTVAAPSVFIFPPSDEQLKSGTASVVCLLNNFYPREAKVQWKVDNALQSGNSQESVTEQDSKDSTYSLSSTLTLSKADYEKHKVYACEVTHQGLSSPVTKSFNRGEC

SEQ ID NO: 9 - protein, 447 aa, Artificial Sequence
  bispecific IgG1 antibody, heavy chain B
EVMLVESGGGLVKPGGSLKLSCAASGFTFSSYTMSWVRQTPEKRLEWVATISSGGDNTYYPDSVKGRFTISRDNAKNNLYLQMSSLRSEDTALYYCARFDYGSSLDCWGQGTTLTVSSASTKGPSVFPLAPSSKSTSGGTAALGCLVKDYFPEPVTVSWNSGALTSGVHTFPAVLQSSGLYSLSSVVTVPSSSLGTQTYICNVNHKPSNTKVDKKVEPKSCDKTHTCPPCPAPELLGGPSVFLFPPKPKDTLMISRTPEVTCVVVDVSHEDPEVKFNWYVDGVEVHNAKTKPREEQYNSTYRVVSVLTVLHQDWLNGKEYKCKVSNKALPAPIEKTISKAKGQPREPQVYTLPPCRDELTKNQVSLWCLVKGFYPSDIAVEWESNGQPENNYKTTPPVLDSDGSFFLYSKLTVDKSRWQQGNVFSCSVMHEALHNRFTQKSLSLSPG

SEQ ID NO: 10 - protein, 225 aa, Artificial Sequence
  bispecific IgG1 antibody, light chain A
DIVLTQSPASLAVSLGQRATISCRASESVDSYGQSYMHWYQQKAGQPPKLLIYLASNLESGVPARFSGSGSRTDFTLTIDPVQAEDAATYYCQQNAEDSRTFGGGTKLEIKRTVIAELPPKVSVFVPPRDGFFGNPRKSKLICQATGFSPRQIQVSWLREGKQVGSGVTTDQVQAEAKESGPTTYKVTSTLTIKESDWLGQSMFTCRVDHRGLTFQQQASSMCVP

SEQ ID NO: 11 - protein, 467 aa, Artificial Sequence
  bispecific IgG1 antibody, heavy chain A
EVQLKESGPGLVAPGGSLSITCTVSGFSLTDSSINWVRQPPGKGLEWLGMIWGDGRIDYADALKSRLSISKDSSKSQVFLEMTSLRTDDTATYYCARDGYFPYAMDFWGQGTSVTVSSASTKGPVIAELPPKVSVFVPPRDGFFGNPRKSKLICQATGFSPRQIQVSWLREGKQVGSGVTTDQVQAEAKESGPTTYKVTSTLTIKESDWLGQSMFTCRVDHRGLTFQQQASSMCVPEPKSADKTHTCPPCPAPELLGGPSVFLFPPKPKDTLMISRTPEVTCVVVDVSHEDPEVKFNWYVDGVEVHNAKTKPREEQYNSTYRVVSVLTVLHQDWLNGKEYKCKVSNKALPAPIEKTISKAKGQPREPQVCTLPPSRDELTKNQVSLSCAVKGFYPSDIAVEWESNGQPENNYKTTPPVLDSDGSFFLVSKLTVDKSRWQQGNVFSCSVMHEALHNHYTQKSLSLSPG

SEQ ID NO: 12 - protein, 214 aa, Artificial Sequence
  bispecific IgG1 antibody, light chain B
DIQMTQSPASLSVSVGDTITLTCHASQNIDVWLSWFQQKPGNIPKLLIYKASNLHTGVPSRFSGSGSGTGFTLTISSLQPEDIATYYCQQAHSYPFTFGGGTKLEIKRTVAAPSVFIFPPSDEQLKSGTASVVCLLNNFYPREAKVQWKVDNALQSGNSQESVTEQDSKDSTYSLSSTLTLSKADYEKHKVYACEVTHQGLSSPVTKSFNRGEC

SEQ ID NO: 13 - protein, 452 aa, Artificial Sequence
  bispecific IgG1 antibody, heavy chain B
QVQLQQSGPELVKPGASVKISCKASGYSFTSYWIHWIKQRPGQGLEWIGMIDPSDGETRLNQRFQGRATLTVDESTSTAYMQLRSPTSEDSAVYYCTRLKEYGNYDSFYFDVWGAGTLVTVSSASTKGPSVFPLAPSSKSTSGGTAALGCLVKDYFPEPVTVSWNSGALTSGVHTFPAVLQSSGLYSLSSVVTVPSSSLGTQTYICNVNHKPSNTKVDKKVEPKSCDKTHTCPPCPAPELLGGPSVFLFPPKPKDTLMISRTPEVTCVVVDVSHEDPEVKFNWYVDGVEVHNAKTKPREEQYNSTYRVVSVLTVLHQDWLNGKEYKCKVSNKALPAPIEKTISKAKGQPREPQVYTLPPCRDELTKNQVSLWCLVKGFYPSDIAVEWESNGQPENNYKTTPPVLDSDGSFFLYSKLTVDKSRWQQGNVFSCSVMHEALHNRFTQKSLSLSPG

SEQ ID NO: 14 - protein, 226 aa, Artificial Sequence
  bivalent Fab, light chain A
DIVMTQTPLSLSVTPGQPASISCKSSQSLVHNNANTYLSWYLQKPGQSPQSLIYKVSNRFSGVPDRFSGSGSGTDFTLKISRVEAEDVGVYYCGQGTQYPFTFGSGTKVEIKRTVIAELPPKVSVFVPPRDGFFGNPRKSKLICQATGFSPRQIQVSWLREGKQVGSGVTTDQVQAEAKESGPTTYKVTSTLTIKESDWLGQSMFTCRVDHRGLTFQQNASSMCVP

SEQ ID NO: 15 - protein, 473 aa, Artificial Sequence
  bivalent Fab, heavy chain
QVQLVESGGGVVQPGRSLRLSCAASGFTFTKAWMHWVRQAPGKQLEWVAQIKDKSNSYATYYADSVKGRFTISRDDSKNTLYLQMNSLRAEDTAVYYCRGVYYALSPFDYWGQGTLVTVSSGGVIAELPPKVSVFVPPRDGFFGNPRKSKLICQATGFSPRQIQVSWLREGKQVGSGVTTDQVQAEAKESGPTTYKVTSTLTIKESDWLGQSMFTCRVDHRGLTFQQNASSMCVPGGGSEVQLVQSGAEVKKPGESLKISCKGSGYSFTDYYMKWARQMPGKGLEWMGDIIPSSGATFYNQKFKGQVTISADKSISTTYLQWSSLKASDTAMYYCARSHLLRASWFAYWGQGTMVTVSSASTKGPSVFPLAPSSKSTSGGTAALGCLVKDYFPEPVTVSWNSGALTSGVHTFPAVLQSSGLYSLSSVVTVPSSSLGTQTYICNVNHKPSNTKVDKKVEPKSCDKTHTHHHHHH

SEQ ID NO: 16 - protein, 220 aa, Artificial Sequence; identical to SEQ ID NO: 3
  bivalent Fab, light chain B

SEQ ID NO: 17 - protein, 226 aa, Artificial Sequence; identical to SEQ ID NO: 14
  bivalent bispecific antibody, light chain LC1

SEQ ID NO: 18 - protein, 685 aa, Artificial Sequence
  bivalent bispecific antibody, heavy chain HC1
QVQLVESGGGVVQPGRSLRLSCAASGFTFTKAWMHWVRQAPGKQLEWVAQIKDKSNSYATYYADSVKGRFTISRDDSKNTLYLQMNSLRAEDTAVYYCRGVYYALSPFDYWGQGTLVTVSSGGVIAELPPKVSVFVPPRDGFFGNPRKSKLICQATGFSPRQIQVSWLREGKQVGSGVTTDQVQAEAKESGPTTYKVTSTLTIKESDWLGQSMFTCRVDHRGLTFQQNASSMCVPGGGSEVQLVQSGAEVKKPGESLKISCKGSGYSFTDYYMKWARQMPGKGLEWMGDIIPSSGATFYNQKFKGQVTISADKSISTTYLQWSSLKASDTAMYYCARSHLLRASWFAYWGQGTMVTVSSASTKGPSVFPLAPCSRSTSESTAALGCLVKDYFPEPVTVSWNSGALTSGVHTFPAVLQSSGLYSLSSVVTVPSSSLGTKTYTCNVDHKPSNTKVDKRVESKYGPPCPPCPAPEFEGGPSVFLFPPKPKDTLMISRTPEVTCVVVDVSQEDPEVQFNWYVDGVEVHNAKTKPREEQFNSTYRVVSVLTVLHQDWLNGKEYKCKVSNKGLPSSIEKTISKAKGQPREPQVYTLPPSQEEMTKNQVSLTCLVKGFYPSDIAVEWESNGQPENNYKTTPPVLDSDGSFFLYSRLTVDKSRWQEGNVFSCSVMHEALHNHYTQKSLSLSLG

SEQ ID NO: 19 - protein, 448 aa, Artificial Sequence
  bivalent bispecific antibody, light chain LC2
DIVMTQSPDSLAVSLGERATINCESSQSLLNSGNQKNYLTWYQQKPGQPPKPLIYWASTRESGVPDRFSGSGSGTDFTLTISSLQAEDVAVYYCQNDYSYPYTFGQGTKLEIKRTVAAPSVFIFPPSDEQLKSGTASVVCLLNNFYPREAKVQWKVDNALQSGNSQESVTEQDSKDSTYSLSSTLTLSKADYEKHKVYACEVTHQGLSSPVTKSFNRGECESKYGPPCPPCPAPEFEGGPSVFLFPPKPKDTLMISRTPEVTCVVVDVSQEDPEVQFNWYVDGVEVHNAKTKPREEQFNSTYRVVSVLTVLHQDWLNGKEYKCKVSNKGLPSSIEKTISKAKGQPREPQVYTLPPSQEEMTKNQVSLTCLVKGFYPSDIAVEWESNGQPENNYKTTPPVLDSDGSFFLYSRLTVDKSRWQEGNVFSCSVMHEALHNRFTQKSLSLSLG

SEQ ID NO: 20 - protein, 367 aa, Artificial Sequence
  CH2E-pseudo-CODV antibody, chain 1
EVQLKESGPGLVAPGGSLSITCTVSGFSLTDSSINWVRQPPGKGLEWLGMIWGDGRIDYADALKSRLSISKDSSKSQVFLEMTSLRTDDTATYYCARDGYFPYAMDFWGQGTSVTVSSSQVQLQQSGPELVKPGASVKISCKASGYSFTSYWIHWIKQRPGQGLEWIGMIDPSDGETRLNQRFQGRATLTVDESTSTAYMQLRSPTSEDSAVYYCTRLKEYGNYDSFYFDVWGAGTLVTVSSRTASTKGPVASRDFTPPTVKILQSSCDGGGHFPPTIQLLCLVSGYTPGTIQITWLEDGQVMDVDLSTASTTQEGELASTQSELTLSQKHWLSDRTYTCQVTYQGHTFEDSTKKCAGSHHHHHHHH

SEQ ID NO: 21 - protein, 339 aa, Artificial Sequence
  CH2E-pseudo-CODV antibody, chain 2
DIQMTQSPASLSVSVGDTITLTCHASQNIDVWLSWFQQKPGNIPKLLIYKASNLHTGVPSRFSGSGSGTGFTLTISSLQPEDIATYYCQQAHSYPFTFGGGTKLEIKGQPKAAPDIVLTQSPASLAVSLGQRATISCRASESVDSYGQSYMHWYQQKAGQPPKLLIYLASNLESGVPARFSGSGSRTDFTLTIDPVQAEDAATYYCQQNAEDSRTFGGGTKLEIKTKGPSRTVASRDFTPPTVKILQSSCDGGGHFPPTIQLLCLVSGYTPGTIQITWLEDGQVMDVDLSTASTTQEGELASTQSELTLSQKHWLSDRTYTCQVTYQGHTFEDSTKKCA

SEQ ID NO: 22 - protein, 338 aa, Artificial Sequence
  pseudo hinge-CH2E-hybrid-Fab2, heavy chain A
VQLQQSGPELVKPGASVKISCKASGYSFTSYWIHWIKQRPGQGLEWIGMIDPSDGETRLNQRFQGRATLTVDESTSTAYMQLRSPTSEDSAVYYCTRLKEYGNYDSFYFDVWGAGTLVTVSSASTKGPSVFPLAPSSKSTSGGTAALGCLVKDYFPEPVTVSWNSGALTSGVHTFPAVLQSSGLYSLSSVVTVPSSSLGTQTYICNVNHKPSNTKVDKKVEPKSCGSGSGSVASRDFTPPTVKILQSSCDGGGHFPPTIQLLCLVSGYTPGTIQITWLEDGQVMDVDLSTASTTQEGELASTQSELTLSQKHWLSDRTYTCQVTYQGHTFEDSTKKCA

SEQ ID NO: 23 - protein, 214 aa, Artificial Sequence; identical to SEQ ID NO: 12
  pseudo hinge-CH2E-hybrid-Fab2, light chain A

SEQ ID NO: 24 - protein, 359 aa, Artificial Sequence
  pseudo hinge-CH2E-hybrid-Fab2, heavy chain B
EVQLKESGPGLVAPGGSLSITCTVSGFSLTDSSINWVRQPPGKGLEWLGMIWGDGRIDYADALKSRLSISKDSSKSQVFLEMTSLRTDDTATYYCARDGYFPYAMDFWGQGTSVTVSSGSGSGSVIAELPPKVSVFVPPRDGFFGNPRKSKLICQATGFSPRQIQVSWLREGKQVGSGVTTDQVQAEAKESGPTTYKVTSTLTIKESDWLGQSMFTCRVDHRGLTFQQQASSMCVPGSGSGSVASRDFTPPTVKILQSSCDGGGHFPPTIQLLCLVSGYTPGTIQITWLEDGQVMDVDLSTASTTQEGELASTQSELTLSQKHWLSDRTYTCQVTYQGHTFEDSTKKCAGSHHHHHHHH

SEQ ID NO: 25 - protein, 225 aa, Artificial Sequence; identical to SEQ ID NO: 10
  pseudo hinge-CH2E-hybrid-Fab2, light chain B

SEQ ID NO: 26 - protein, 214 aa, Artificial Sequence; identical to SEQ ID NO: 12
  bispecific IgG1 antibody, light chain A

SEQ ID NO: 27 - protein, 443 aa, Artificial Sequence
  bispecific IgG1 antibody, heavy chain A
QVQLQQSGPELVKPGASVKISCKASGYSFTSYWIHWIKQRPGQGLEWIGMIDPSDGETRLNQRFQGRATLTVDESTSTAYMQLRSPTSEDSAVYYCTRLKEYGNYDSFYFDVWGAGTLVTVSSASTKGPSVFPLAPSSKSTSGGTAALGCLVKDYFPEPVTVSWNSGALTSGVHTFPAVLQSSGLYSLSSVVTVPSSSLGTQTYICNVNHKPSNTKVDKTHTCPPCPAPEAAGGPSVFLFPPKPKDTLMISRTPEVTCVVVDVSHEDPEVKFNWYVDGVEVHNAKTKPREEQYNSTYRVVSVLTVLHQDWLNGKEYKCKVSNKALPAPIEKTISKAKGQPREPQVYTLPPCRDELTKNQVSLWCLVKGFYPSDIAVEWESNGQPENNYKTTPPVLDSDGSFFLYSKLTVDKSRWQQGNVFSCSVMHEALHNRFTQKSLSLSPG

SEQ ID NO: 28 - protein, 220 aa, Artificial Sequence
  bispecific IgG1 antibody, light chain B
DIVLTQSPASLAVSLGQRATISCRASESVDSYGQSYMHWYQQKAGQPPKLLIYLASNLESGVPARFSGSGSRTDFTLTIDPVQAEDAATYYCQQNAEDSRTFGGGTKLEIKRTVASRDFTPPTVKILQSSCDGGGHFPPTIQLLCLVSGYTPGTIQITWLEDGQVMDVDLSTASTTQEGELASTQSELTLSQKHWLSDRTYTCQVTYQGHTFEDSTKKCA

SEQ ID NO: 29 - protein, 463 aa, Artificial Sequence
  bispecific IgG1 antibody, heavy chain B
EVQLKESGPGLVAPGGSLSITCTVSGFSLTDSSINWVRQPPGKGLEWLGMIWGDGRIDYADALKSRLSISKDSSKSQVFLEMTSLRTDDTATYYCARDGYFPYAMDFWGQGTSVTVSSGSGSGSVASRDFTPPTVKILQSSCDGGGHFPPTIQLLCLVSGYTPGTIQITWLEDGQVMDVDLSTASTTQEGELASTQSELTLSQKHWLSDRTYTCQVTYQGHTFEDSTKKCAGSGSGSDKTHTCPPCPAPEAAGGPSVFLFPPKPKDTLMISRTPEVTCVVVDVSHEDPEVKFNWYVDGVEVHNAKTKPREEQYNSTYRVVSVLTVLHQDWLNGKEYKCKVSNKALPAPIEKTISKAKGQPREPQVCTLPPSRDELTKNQVSLSCAVKGFYPSDIAVEWESNGQPENNYKTTPPVLDSDGSFFLVSKLTVDKSRWQQGNVFSCSVMHEALHNHYTQKSLSLSPG

SEQ ID NO: 30 - protein, 225 aa, Artificial Sequence; identical to SEQ ID NO: 10
  Trispecific antibody, light chain A

SEQ ID NO: 31 - protein, 463 aa, Artificial Sequence
  Trispecific antibody, heavy chain A
EVQLKESGPGLVAPGGSLSITCTVSGFSLTDSSINWVRQPPGKGLEWLGMIWGDGRIDYADALKSRLSISKDSSKSQVFLEMTSLRTDDTATYYCARDGYFPYAMDFWGQGTSVTVSSASTKGPVIAELPPKVSVFVPPRDGFFGNPRKSKLICQATGFSPRQIQVSWLREGKQVGSGVTTDQVQAEAKESGPTTYKVTSTLTIKESDWLGQSMFTCRVDHRGLTFQQQASSMCVPDKTHTCPPCPAPELLGGPSVFLFPPKPKDTLMISRTPEVTCVVVDVSHEDPEVKFNWYVDGVEVHNAKTKPREEQYNSTYRVVSVLTVLHQDWLNGKEYKCKVSNKALPAPIEKTISKAKGQPREPQVCTLPPSRDELTKNQVSLSCAVKGFYPSDIAVEWESNGQPENNYKTTPPVLDSDGSFFLVSKLTVDKSRWQQGNVFSCSVMHEALHNRFTQKSLSLSPGK

SEQ ID NO: 32 - protein, 340 aa, Artificial Sequence
  Trispecific antibody, light chain B
DIQMTQSPASLSVSVGDTITLTCHASQNIDVWLSWFQQKPGNIPKLLIYKASNLHTGVPSRFSGSGSGTGFTLTISSLQPEDIATYYCQQAHSYPFTFGGGTKLEIKGGSGSSGSGGDIQMTQSPSSLSASVGDRVTITCRASQGIRNYLAWYQQKPGKAPKLLIYAASTLQSGVPSRFSGSGSGTDFTLTISSLQPEDVATYYCQRYNRAPYTFGQGTKVEIKGGSGSSGSGGGQPKAAPSVTLFPPSSEELQANKATLVCLISDFYPGAVTVAWKADSSPVKAGVETTTPSKQSNNKYAASSYLSLTPEQWKSHRSYSCQVTHEGSTVEKTVAPTECS

SEQ ID NO: 33 - protein, 573 aa, Artificial Sequence
  Trispecific antibody, heavy chain B
EVQLVESGGGLVQPGRSLRLSCAASGFTFDDYAMHWVRQAPGKGLEWVSAITWNSGHIDYADSVEGRFTISRDNAKNSLYLQMNSLRAEDTAVYYCAKVSYLSTASSLDYWGQGTLVTVSSQVQLQQSGPELVKPGASVKISCKASGYSFTSYWIHWIKQRPGQGLEWIGMIDPSDGETRLNQRFQGRATLTVDESTSTAYMQLRSPTSEDSAVYYCTRLKEYGNYDSFYFDVWGAGTLVTVSSASTKGPSVFPLAPSSKSTSGGTAALGCLVKDYFPEPVTVSWNSGALTSGVHTFPAVLQSSGLYSLSSVVTVPSSSLGTQTYICNVNHKPSNTKVDKKVEPKSCDKTHTCPPCPAPELLGGPSVFLFPPKPKDTLMISRTPEVTCVVVDVSHEDPEVKFNWYVDGVEVHNAKTKPREEQYNSTYRVVSVLTVLHQDWLNGKEYKCKVSNKALPAPIEKTISKAKGQPREPQVYTLPPCRDELTKNQVSLWCLVKGFYPSDIAVEWESNGQPENNYKTTPPVLDSDGSFFLYSKLTVDKSRWQQGNVFSCSVMHEALHNHYTQKSLSLSPG